European Patent Application EP 4 495 140 A1, published January 22, 2025. Title: CLAUDIN18.2 HUMANIZED ANTIBODY AND APPLICATION THEREOF. Applicant: SUNSHINE LAKE PHARMA CO., LTD. Application CN. The sequence listing filed with the application follows.

SEQUENCE LISTING (112 sequences)

SEQ ID NO: 1 - protein, 17 aa, synthetic construct
  source 1..17: note = X=K or R
XSSQSLFNSGNQKNYLT

SEQ ID NO: 2 - protein, 7 aa, synthetic construct
WASTRES

SEQ ID NO: 3 - protein, 9 aa, synthetic construct
QNDYSYPLT

SEQ ID NO: 4 - protein, 5 aa, synthetic construct
DYNMH

SEQ ID NO: 5 - protein, 17 aa, synthetic construct
  VARIANT 12: note = X=N or S
  VARIANT 16: note = X=K or Q
YINPNNGGTSYXQKFXG

SEQ ID NO: 6 - protein, 6 aa, synthetic construct
TRYLAV

SEQ ID NO: 7 - protein, 17 aa, synthetic construct
  source 1..17: note = X=K or R
XSSQSLLNSGNQKNYLT

SEQ ID NO: 8 - protein, 7 aa, synthetic construct
WASTRES

SEQ ID NO: 9 - protein, 9 aa, synthetic construct
QNDYSYPFT

SEQ ID NO: 10 - protein, 5 aa, synthetic construct
SYWMH

SEQ ID NO: 11 - protein, 17 aa, synthetic construct
  VARIANT 12: note = X=N or A
  VARIANT 13: note = X=E or Q
  VARIANT 16: note = X=K or Q
  VARIANT 17: note = X=S or G
MIHPNSGSTNYXXKFXX

SEQ ID NO: 12 - protein, 10 aa, synthetic construct
RYYGSISPDY

SEQ ID NO: 13 - protein, 24 aa, synthetic construct
  VARIANT 3: note = X=V or Q
  VARIANT 12: note = X= S or T
  VARIANT 13: note = X=V or A
  VARIANT 14: note = X=T or S
  VARIANT 15: note = X=A or V
  VARIANT 17: note = X=E or D
  VARIANT 18: note = X=K or R
  VARIANT 21: note = X=M or I
  VARIANT 23: note = X=S or T
DIXMTQSPSSLXXXXGXXVTXSXC

SEQ ID NO: 14 - protein, 15 aa, synthetic construct
  VARIANT 8: note = X=Q or K
  VARIANT 9: note = X=P or A
WYQQKPGXXPKLLIY

SEQ ID NO: 15 - protein, 33 aa, synthetic construct
  VARIANT 4: note = X=D or S
  VARIANT 8: note = X=T or S
  VARIANT 23: note = X=V or L
  VARIANT 25: note = X=A or P
  VARIANT 28: note = X=L or F
  VARIANT 30: note = X=V or T
  VARIANT 32: note = X=F or Y
GVPXDRFXGSGSGTDFTLTISSXQXEDXAXYXC

SEQ ID NO: 16 - protein, 10 aa, synthetic construct
  VARIANT 3: note = X=A or G
  VARIANT 9: note = X=L or I
FGXGTKLEXK

SEQ ID NO: 17 - protein, 30 aa, synthetic construct
  VARIANT 1: note = X=E or Q
  VARIANT 5: note = X=Q or V
  VARIANT 9: note = X=P or A
  VARIANT 11: note = X=L or V
  VARIANT 12: note = X=V or K
  VARIANT 13: note = X=R or K
  VARIANT 20: note = X=M or V
XVQLXQSGXEXXXPGASVKXSCKASGYTFT

SEQ ID NO: 18 - protein, 14 aa, synthetic construct
  VARIANT 3: note = X=K or R
  VARIANT 5: note = X=S or A
  VARIANT 6: note = X=H or P
  VARIANT 8: note = X=K or Q
  VARIANT 9: note = X=S or R
  VARIANT 13: note = X=I or M
WVXQXXGXXLEWXG

SEQ ID NO: 19 - protein, 32 aa, synthetic construct
  VARIANT 1: note = X=K or R
  VARIANT 2: note = X=A or V
  VARIANT 4: note = X=L or I
  VARIANT 6: note = X=V or R
  VARIANT 7: note = X=N or D
  VARIANT 8: note = X=K or T
  VARIANT 10: note = X=S or A
  VARIANT 18: note = X=R or S
  VARIANT 21: note = X=T or R
  VARIANT 25: note = X=S or T
XXTXTXXXSXSTAYMELXSLXSEDXAVYYCVT

SEQ ID NO: 20 - protein, 11 aa, synthetic construct
  source 1..11: note = X=T or Q
WGXGTTVTVSS

SEQ ID NO: 21 - protein, 24 aa, synthetic construct
  VARIANT 3: note = X=V or Q
  VARIANT 13: note = X=V or A
  VARIANT 14: note = X=T or S
  VARIANT 16: note = X=A or V
  VARIANT 18: note = X=E or D
  VARIANT 19: note = X=K or R
  VARIANT 22: note = X=M or I
  VARIANT 23: note = X=S or T
DIXMTQSPSSLSXXAXGXXVTXXC

SEQ ID NO: 22 - protein, 15 aa, synthetic construct
  VARIANT 8: note = X=Q or K
  VARIANT 9: note = X=P or A
WYQQKPGXXPKLLIY

SEQ ID NO: 23 - protein, 32 aa, synthetic construct
  VARIANT 4: note = X=D or S
  VARIANT 7: note = X=T or S
  VARIANT 22: note = X=V or L
  VARIANT 24: note = X=A or P
  VARIANT 27: note = X=L or F
  VARIANT 29: note = X=V or T
GVPXRFXGSGSGTDFTLTISSXQXEDXAXYYC

SEQ ID NO: 24 - protein, 10 aa, synthetic construct
  source 1..10: note = X=S or G
FGXGTKLEIK

SEQ ID NO: 25 - protein, 30 aa, synthetic construct
  VARIANT 5: note = X=Q or V
  VARIANT 7: note = X=P or S
  VARIANT 9: note = X=S or A
  VARIANT 11: note = X=L or V
  VARIANT 12: note = X=V or K
  VARIANT 20: note = X=L or V
QVQLXQXGXEXXKPGASVKXSCKASGYTFT

SEQ ID NO: 26 - protein, 14 aa, synthetic construct
  VARIANT 3: note = X=K or R
  VARIANT 5: note = X=R or A
  VARIANT 13: note = X=I or M
WVXQXPGQGLEWXG

SEQ ID NO: 27 - protein, 33 aa, synthetic construct
  VARIANT 1: note = X=S or G
  VARIANT 2: note = X=R or K
  VARIANT 3: note = X=A or V
  VARIANT 5: note = X=L or M
  VARIANT 9: note = X=K or T
  VARIANT 11: note = X=S or T
  VARIANT 14: note = X=A or V
  VARIANT 17: note = X=Q or E
  VARIANT 22: note = X=T or R
  VARIANT 26: note = X=S or T
XXXTXTVDXSXSTXYMXLSSLXSEDXAVYYCAR

SEQ ID NO: 28 - protein, 11 aa, synthetic construct
  source 1..11: note = X=L or V
WGQGTTXTVSS

SEQ ID NO: 29 - protein, 17 aa, synthetic construct
KSSQSLFNSGNQKNYLT

SEQ ID NO: 30 - protein, 7 aa, synthetic construct
WASTRES

SEQ ID NO: 31 - protein, 9 aa, synthetic construct
QNDYSYPLT

SEQ ID NO: 32 - protein, 5 aa, synthetic construct
DYNMH

SEQ ID NO: 33 - protein, 17 aa, synthetic construct
YINPNNGGTSYNQKFKG

SEQ ID NO: 34 - protein, 6 aa, synthetic construct
TRYLAV

SEQ ID NO: 35 - protein, 17 aa, synthetic construct
KSSQSLLNSGNQKNYLT

SEQ ID NO: 36 - protein, 7 aa, synthetic construct
WASTRES

SEQ ID NO: 37 - protein, 9 aa, synthetic construct
QNDYSYPFT

SEQ ID NO: 38 - protein, 5 aa, synthetic construct
SYWMH

SEQ ID NO: 39 - protein, 17 aa, synthetic construct
MIHPNSGSTNYNEKFKS

SEQ ID NO: 40 - protein, 10 aa, synthetic construct
RYYGSISPDY

SEQ ID NO: 41 - protein, 23 aa, synthetic construct
  VARIANT 3: note = X=V or Q
  VARIANT 13: note = X=V or A
  VARIANT 21: note = X=M or I
DIXMTQSPSSLSXTAGEKVTXSC

SEQ ID NO: 42 - protein, 15 aa, synthetic construct
WYQQKPGQPPKLLIY

SEQ ID NO: 43 - protein, 33 aa, synthetic construct
  VARIANT 4: note = X=D or S
  VARIANT 23: note = X=V or L
  VARIANT 32: note = X=F or Y
GVPXDRFTGSGSGTDFTLTISSXQAEDLAVYXC

SEQ ID NO: 44 - protein, 10 aa, synthetic construct
FGAGTKLELK

SEQ ID NO: 45 - protein, 30 aa, synthetic construct
  VARIANT 1: note = X=E or Q
  VARIANT 20: note = X=M or V
XVQLQQSGPELVRPGASVKXSCKASGYTFT

SEQ ID NO: 46 - protein, 14 aa, synthetic construct
  VARIANT 8: note = X=K or Q
  VARIANT 9: note = X=S or R
  VARIANT 13: note = X=I or M
WVKQSHGXXLEWXG

SEQ ID NO: 47 - protein, 32 aa, synthetic construct
  VARIANT 1: note = X=K or R
  VARIANT 2: note = X=A or V
  VARIANT 4: note = X=L or I
  VARIANT 7: note = X=N or D
  VARIANT 8: note = X=K or T
  VARIANT 10: note = X=S or A
XXTXTVXXSXSTAYMELRSLTSEDSAVYYCVT

SEQ ID NO: 48 - protein, 11 aa, synthetic construct
WGTGTTVTVSS

SEQ ID NO: 49 - protein, 23 aa, synthetic construct
  VARIANT 3: note = X=V or Q
  VARIANT 13: note = X=V or A
  VARIANT 21: note = X=M or I
DIXMTQSPSSLSXTAGEKVTXSC

SEQ ID NO: 50 - protein, 15 aa, synthetic construct
  VARIANT 8: note = X=Q or K
  VARIANT 9: note = X=P or A
WYQQKPGXXPKLLIY

SEQ ID NO: 51 - protein, 32 aa, synthetic construct
  VARIANT 4: note = X=D or S
  VARIANT 22: note = X=V or L
GVPXRFTGSGSGTDFTLTISSXQAEDLAVYYC

SEQ ID NO: 52 - protein, 10 aa, synthetic construct
FGSGTKLEIK

SEQ ID NO: 53 - protein, 30 aa, synthetic construct
  source 1..30: note = X=L or V
QVQLQQPGSELVKPGASVKXSCKASGYTFT

SEQ ID NO: 54 - protein, 14 aa, synthetic construct
  VARIANT 5: note = X=R or A
  VARIANT 13: note = X=I or M
WVKQXPGQGLEWXG

SEQ ID NO: 55 - protein, 32 aa, synthetic construct
  VARIANT 1: note = X=R or K
  VARIANT 2: note = X=A or V
  VARIANT 4: note = X=L or M
  VARIANT 8: note = X=K or T
  VARIANT 13: note = X=A or V
XXTXTVDXSSSTXYMQLSSLTSEDSAVYYCAR

SEQ ID NO: 56 - protein, 11 aa, synthetic construct
WGQGTTLTVSS

SEQ ID NO: 57 - protein, 113 aa, synthetic construct
DIVMTQSPSSLSVSVGDRVTMTCKSSQSLFNSGNQKNYLTWYQQKPGKAPKLLIYWASTRESGVPDRFSGSGSGTDFTLTISSVQPEDFATYFCQNDYSYPLTFGGGTKLEIK

SEQ ID NO: 58 - protein, 113 aa, synthetic construct
DIQMTQSPSSLSASVGDRVTMTCKSSQSLFNSGNQKNYLTWYQQKPGKAPKLLIYWASTRESGVPSRFSGSGSGTDFTLTISSLQPEDFATYYCQNDYSYPLTFGGGTKLEIK

SEQ ID NO: 59 - protein, 113 aa, synthetic construct
DIQMTQSPSSLSASVGDRVTITCRSSQSLFNSGNQKNYLTWYQQKPGKAPKLLIYWASTRESGVPSRFSGSGSGTDFTLTISSLQPEDFATYYCQNDYSYPLTFGGGTKLEIK

SEQ ID NO: 60 - protein, 115 aa, synthetic construct
EVQLVQSGAEVKKPGASVKMSCKASGYTFTDYNMHWVRQAPGKSLEWIGYINPNNGGTSYNQKFKGKATLTVNKSSSTAYMELSSLRSEDTAVYYCVTTRYLAVWGQGTTVTVSS

SEQ ID NO: 61 - protein, 115 aa, synthetic construct
QVQLVQSGAEVKKPGASVKMSCKASGYTFTDYNMHWVRQAPGQRLEWIGYINPNNGGTSYNQKFKGKATLTVDTSASTAYMELSSLRSEDTAVYYCVTTRYLAVWGQGTTVTVSS

SEQ ID NO: 62 - protein, 115 aa, synthetic construct
QVQLVQSGAEVKKPGASVKVSCKASGYTFTDYNMHWVRQAPGQRLEWIGYINPNNGGTSYNQKFKGRVTITVDTSASTAYMELSSLRSEDTAVYYCVTTRYLAVWGQGTTVTVSS

SEQ ID NO: 63 - protein, 115 aa, synthetic construct
QVQLVQSGAEVKKPGASVKVSCKASGYTFTDYNMHWVRQAPGQRLEWMGYINPNNGGTSYNQKFQGRVTITVDTSASTAYMELSSLRSEDTAVYYCVTTRYLAVWGQGTTVTVSS

SEQ ID NO: 64 - protein, 115 aa, synthetic construct
QVQLVQSGAEVKKPGASVKVSCKASGYTFTDYNMHWVRQAPGQRLEWMGYINPNNGGTSYSQKFQGRVTITRDTSASTAYMELSSLRSEDTAVYYCVTTRYLAVWGQGTTVTVSS

SEQ ID NO: 65 - protein, 113 aa, synthetic construct
DIVMTQSPSSLSVSVGDRVTMTCKSSQSLLNSGNQKNYLTWYQQKPGQPPKLLIYWASTRESGVPDRFSGSGSGTDFTLTISSVQPEDFATYYCQNDYSYPFTFGGGTKLEIK

SEQ ID NO: 66 - protein, 113 aa, synthetic construct
DIQMTQSPSSLSASVGDRVTMTCKSSQSLLNSGNQKNYLTWYQQKPGKAPKLLIYWASTRESGVPSRFSGSGSGTDFTLTISSLQPEDFATYYCQNDYSYPFTFGGGTKLEIK

SEQ ID NO: 67 - protein, 113 aa, synthetic construct
DIQMTQSPSSLSASVGDRVTITCRSSQSLLNSGNQKNYLTWYQQKPGKAPKLLIYWASTRESGVPSRFSGSGSGTDFTLTISSLQPEDFATYYCQNDYSYPFTFGGGTKLEIK

SEQ ID NO: 68 - protein, 119 aa, synthetic construct
QVQLVQSGAEVKKPGASVKLSCKASGYTFTSYWMHWVRQRPGQGLEWIGMIHPNSGSTNYNEKFKSKATLTVDKSTSTAYMELSSLRSEDTAVYYCARRYYGSISPDYWGQGTTVTVSS

SEQ ID NO: 69 - protein, 119 aa, synthetic construct
QVQLVQSGAEVKKPGASVKLSCKASGYTFTSYWMHWVRQAPGQGLEWIGMIHPNSGSTNYNEKFKSRATLTVDTSTSTAYMELSSLRSEDTAVYYCARRYYGSISPDYWGQGTTVTVSS

SEQ ID NO: 70 - protein, 119 aa, synthetic construct
QVQLVQSGAEVKKPGASVKVSCKASGYTFTSYWMHWVRQAPGQGLEWIGMIHPNSGSTNYNEKFKSRVTMTVDTSTSTAYMELSSLRSEDTAVYYCARRYYGSISPDYWGQGTTVTVSS

SEQ ID NO: 71 - protein, 119 aa, synthetic construct
QVQLVQSGAEVKKPGASVKVSCKASGYTFTSYWMHWVRQAPGQGLEWMGMIHPNSGSTNYNEKFKSRVTMTVDTSTSTVYMELSSLRSEDTAVYYCARRYYGSISPDYWGQGTTVTVSS

SEQ ID NO: 72 - protein, 119 aa, synthetic construct
QVQLVQSGAEVKKPGASVKVSCKASGYTFTSYWMHWVRQAPGQGLEWMGMIHPNSGSTNYAQKFQGRVTMTRDTSTSTVYMELSSLRSEDTAVYYCARRYYGSISPDYWGQGTTVTVSS

SEQ ID NO: 73 - protein, 107 aa, synthetic construct [sequence omitted]

SEQ ID NO: 74 - protein, 330 aa, synthetic construct [sequence omitted]

SEQ ID NO: 75 - protein, 327 aa, synthetic construct
ASTKGPSVFPLAPCSRSTSESTAALGCLVKDYFPEPVTVSWNSGALTSGVHTFPAVLQSSGLYSLSSVVTVPSSSLGTKTYTCNVDHKPSNTKVDKRVESKYGPPCPPCPAPEFLGGPSVFLFPPKPKDTLMISRTPEVTCVVVDVSQEDPEVQFNWYVDGVEVHNAKTKPREEQFNSTYRVVSVLTVLHQDWLNGKEYKCKVSNKGLPSSIEKTISKAKGQPREPQVYTLPPSQEEMTKNQVSLTCLVKGFYPSDIAVEWESNGQPENNYKTTPPVLDSDGSFFLYSRLTVDKSRWQEGNVFSCSVMHEALHNHYTQKSLSLSLGK

SEQ ID NO: 76 - protein, 220 aa, synthetic construct
DIVMTQSPSSLSVSVGDRVTMTCKSSQSLFNSGNQKNYLTWYQQKPGKAPKLLIYWASTRESGVPDRFSGSGSGTDFTLTISSVQPEDFATYFCQNDYSYPLTFGGGTKLEIKRTVAAPSVFIFPPSDEQLKSGTASVVCLLNNFYPREAKVQWKVDNALQSGNSQESVTEQDSKDSTYSLSSTLTLSKADYEKHKVYACEVTHQGLSSPVTKSFNRGEC

SEQ ID NO: 77 - protein, 220 aa, synthetic construct
DIQMTQSPSSLSASVGDRVTMTCKSSQSLFNSGNQKNYLTWYQQKPGKAPKLLIYWASTRESGVPSRFSGSGSGTDFTLTISSLQPEDFATYYCQNDYSYPLTFGGGTKLEIKRTVAAPSVFIFPPSDEQLKSGTASVVCLLNNFYPREAKVQWKVDNALQSGNSQESVTEQDSKDSTYSLSSTLTLSKADYEKHKVYACEVTHQGLSSPVTKSFNRGEC

SEQ ID NO: 78 - protein, 220 aa, synthetic construct
DIQMTQSPSSLSASVGDRVTITCRSSQSLFNSGNQKNYLTWYQQKPGKAPKLLIYWASTRESGVPSRFSGSGSGTDFTLTISSLQPEDFATYYCQNDYSYPLTFGGGTKLEIKRTVAAPSVFIFPPSDEQLKSGTASVVCLLNNFYPREAKVQWKVDNALQSGNSQESVTEQDSKDSTYSLSSTLTLSKADYEKHKVYACEVTHQGLSSPVTKSFNRGEC

SEQ ID NO: 79 - protein, 445 aa, synthetic construct
EVQLVQSGAEVKKPGASVKMSCKASGYTFTDYNMHWVRQAPGKSLEWIGYINPNNGGTSYNQKFKGKATLTVNKSSSTAYMELSSLRSEDTAVYYCVTTRYLAVWGQGTTVTVSSASTKGPSVFPLAPSSKSTSGGTAALGCLVKDYFPEPVTVSWNSGALTSGVHTFPAVLQSSGLYSLSSVVTVPSSSLGTQTYICNVNHKPSNTKVDKKVEPKSCDKTHTCPPCPAPELLGGPSVFLFPPKPKDTLMISRTPEVTCVVVDVSHEDPEVKFNWYVDGVEVHNAKTKPREEQYNSTYRVVSVLTVLHQDWLNGKEYKCKVSNKALPAPIEKTISKAKGQPREPQVYTLPPSRDELTKNQVSLTCLVKGFYPSDIAVEWESNGQPENNYKTTPPVLDSDGSFFLYSKLTVDKSRWQQGNVFSCSVMHEALHNHYTQKSLSLSPGK

SEQ ID NO: 80 - protein, 445 aa, synthetic construct
QVQLVQSGAEVKKPGASVKMSCKASGYTFTDYNMHWVRQAPGQRLEWIGYINPNNGGTSYNQKFKGKATLTVDTSASTAYMELSSLRSEDTAVYYCVTTRYLAVWGQGTTVTVSSASTKGPSVFPLAPSSKSTSGGTAALGCLVKDYFPEPVTVSWNSGALTSGVHTFPAVLQSSGLYSLSSVVTVPSSSLGTQTYICNVNHKPSNTKVDKKVEPKSCDKTHTCPPCPAPELLGGPSVFLFPPKPKDTLMISRTPEVTCVVVDVSHEDPEVKFNWYVDGVEVHNAKTKPREEQYNSTYRVVSVLTVLHQDWLNGKEYKCKVSNKALPAPIEKTISKAKGQPREPQVYTLPPSRDELTKNQVSLTCLVKGFYPSDIAVEWESNGQPENNYKTTPPVLDSDGSFFLYSKLTVDKSRWQQGNVFSCSVMHEALHNHYTQKSLSLSPGK

SEQ ID NO: 81 - protein, 445 aa, synthetic construct
QVQLVQSGAEVKKPGASVKVSCKASGYTFTDYNMHWVRQAPGQRLEWIGYINPNNGGTSYNQKFKGRVTITVDTSASTAYMELSSLRSEDTAVYYCVTTRYLAVWGQGTTVTVSSASTKGPSVFPLAPSSKSTSGGTAALGCLVKDYFPEPVTVSWNSGALTSGVHTFPAVLQSSGLYSLSSVVTVPSSSLGTQTYICNVNHKPSNTKVDKKVEPKSCDKTHTCPPCPAPELLGGPSVFLFPPKPKDTLMISRTPEVTCVVVDVSHEDPEVKFNWYVDGVEVHNAKTKPREEQYNSTYRVVSVLTVLHQDWLNGKEYKCKVSNKALPAPIEKTISKAKGQPREPQVYTLPPSRDELTKNQVSLTCLVKGFYPSDIAVEWESNGQPENNYKTTPPVLDSDGSFFLYSKLTVDKSRWQQGNVFSCSVMHEALHNHYTQKSLSLSPGK

SEQ ID NO: 82 - protein, 445 aa, synthetic construct
QVQLVQSGAEVKKPGASVKVSCKASGYTFTDYNMHWVRQAPGQRLEWMGYINPNNGGTSYNQKFQGRVTITVDTSASTAYMELSSLRSEDTAVYYCVTTRYLAVWGQGTTVTVSSASTKGPSVFPLAPSSKSTSGGTAALGCLVKDYFPEPVTVSWNSGALTSGVHTFPAVLQSSGLYSLSSVVTVPSSSLGTQTYICNVNHKPSNTKVDKKVEPKSCDKTHTCPPCPAPELLGGPSVFLFPPKPKDTLMISRTPEVTCVVVDVSHEDPEVKFNWYVDGVEVHNAKTKPREEQYNSTYRVVSVLTVLHQDWLNGKEYKCKVSNKALPAPIEKTISKAKGQPREPQVYTLPPSRDELTKNQVSLTCLVKGFYPSDIAVEWESNGQPENNYKTTPPVLDSDGSFFLYSKLTVDKSRWQQGNVFSCSVMHEALHNHYTQKSLSLSPGK

SEQ ID NO: 83 - protein, 445 aa, synthetic construct
QVQLVQSGAEVKKPGASVKVSCKASGYTFTDYNMHWVRQAPGQRLEWMGYINPNNGGTSYSQKFQGRVTITRDTSASTAYMELSSLRSEDTAVYYCVTTRYLAVWGQGTTVTVSSASTKGPSVFPLAPSSKSTSGGTAALGCLVKDYFPEPVTVSWNSGALTSGVHTFPAVLQSSGLYSLSSVVTVPSSSLGTQTYICNVNHKPSNTKVDKKVEPKSCDKTHTCPPCPAPELLGGPSVFLFPPKPKDTLMISRTPEVTCVVVDVSHEDPEVKFNWYVDGVEVHNAKTKPREEQYNSTYRVVSVLTVLHQDWLNGKEYKCKVSNKALPAPIEKTISKAKGQPREPQVYTLPPSRDELTKNQVSLTCLVKGFYPSDIAVEWESNGQPENNYKTTPPVLDSDGSFFLYSKLTVDKSRWQQGNVFSCSVMHEALHNHYTQKSLSLSPGK

SEQ ID NO: 84 - protein, 442 aa, synthetic construct
EVQLVQSGAEVKKPGASVKMSCKASGYTFTDYNMHWVRQAPGKSLEWIGYINPNNGGTSYNQKFKGKATLTVNKSSSTAYMELSSLRSEDTAVYYCVTTRYLAVWGQGTTVTVSSASTKGPSVFPLAPCSRSTSESTAALGCLVKDYFPEPVTVSWNSGALTSGVHTFPAVLQSSGLYSLSSVVTVPSSSLGTKTYTCNVDHKPSNTKVDKRVESKYGPPCPPCPAPEFLGGPSVFLFPPKPKDTLMISRTPEVTCVVVDVSQEDPEVQFNWYVDGVEVHNAKTKPREEQFNSTYRVVSVLTVLHQDWLNGKEYKCKVSNKGLPSSIEKTISKAKGQPREPQVYTLPPSQEEMTKNQVSLTCLVKGFYPSDIAVEWESNGQPENNYKTTPPVLDSDGSFFLYSRLTVDKSRWQEGNVFSCSVMHEALHNHYTQKSLSLSLGK

SEQ ID NO: 85 - protein, 442 aa, synthetic construct
QVQLVQSGAEVKKPGASVKMSCKASGYTFTDYNMHWVRQAPGQRLEWIGYINPNNGGTSYNQKFKGKATLTVDTSASTAYMELSSLRSEDTAVYYCVTTRYLAVWGQGTTVTVSSASTKGPSVFPLAPCSRSTSESTAALGCLVKDYFPEPVTVSWNSGALTSGVHTFPAVLQSSGLYSLSSVVTVPSSSLGTKTYTCNVDHKPSNTKVDKRVESKYGPPCPPCPAPEFLGGPSVFLFPPKPKDTLMISRTPEVTCVVVDVSQEDPEVQFNWYVDGVEVHNAKTKPREEQFNSTYRVVSVLTVLHQDWLNGKEYKCKVSNKGLPSSIEKTISKAKGQPREPQVYTLPPSQEEMTKNQVSLTCLVKGFYPSDIAVEWESNGQPENNYKTTPPVLDSDGSFFLYSRLTVDKSRWQEGNVFSCSVMHEALHNHYTQKSLSLSLGK

SEQ ID NO: 86 - protein, 442 aa, synthetic construct
QVQLVQSGAEVKKPGASVKVSCKASGYTFTDYNMHWVRQAPGQRLEWIGYINPNNGGTSYNQKFKGRVTITVDTSASTAYMELSSLRSEDTAVYYCVTTRYLAVWGQGTTVTVSSASTKGPSVFPLAPCSRSTSESTAALGCLVKDYFPEPVTVSWNSGALTSGVHTFPAVLQSSGLYSLSSVVTVPSSSLGTKTYTCNVDHKPSNTKVDKRVESKYGPPCPPCPAPEFLGGPSVFLFPPKPKDTLMISRTPEVTCVVVDVSQEDPEVQFNWYVDGVEVHNAKTKPREEQFNSTYRVVSVLTVLHQDWLNGKEYKCKVSNKGLPSSIEKTISKAKGQPREPQVYTLPPSQEEMTKNQVSLTCLVKGFYPSDIAVEWESNGQPENNYKTTPPVLDSDGSFFLYSRLTVDKSRWQEGNVFSCSVMHEALHNHYTQKSLSLSLGK

SEQ ID NO: 87 - protein, 442 aa, synthetic construct
QVQLVQSGAEVKKPGASVKVSCKASGYTFTDYNMHWVRQAPGQRLEWMGYINPNNGGTSYNQKFQGRVTITVDTSASTAYMELSSLRSEDTAVYYCVTTRYLAVWGQGTTVTVSSASTKGPSVFPLAPCSRSTSESTAALGCLVKDYFPEPVTVSWNSGALTSGVHTFPAVLQSSGLYSLSSVVTVPSSSLGTKTYTCNVDHKPSNTKVDKRVESKYGPPCPPCPAPEFLGGPSVFLFPPKPKDTLMISRTPEVTCVVVDVSQEDPEVQFNWYVDGVEVHNAKTKPREEQFNSTYRVVSVLTVLHQDWLNGKEYKCKVSNKGLPSSIEKTISKAKGQPREPQVYTLPPSQEEMTKNQVSLTCLVKGFYPSDIAVEWESNGQPENNYKTTPPVLDSDGSFFLYSRLTVDKSRWQEGNVFSCSVMHEALHNHYTQKSLSLSLGK

SEQ ID NO: 88 - protein, 442 aa, synthetic construct
QVQLVQSGAEVKKPGASVKVSCKASGYTFTDYNMHWVRQAPGQRLEWMGYINPNNGGTSYSQKFQGRVTITRDTSASTAYMELSSLRSEDTAVYYCVTTRYLAVWGQGTTVTVSSASTKGPSVFPLAPCSRSTSESTAALGCLVKDYFPEPVTVSWNSGALTSGVHTFPAVLQSSGLYSLSSVVTVPSSSLGTKTYTCNVDHKPSNTKVDKRVESKYGPPCPPCPAPEFLGGPSVFLFPPKPKDTLMISRTPEVTCVVVDVSQEDPEVQFNWYVDGVEVHNAKTKPREEQFNSTYRVVSVLTVLHQDWLNGKEYKCKVSNKGLPSSIEKTISKAKGQPREPQVYTLPPSQEEMTKNQVSLTCLVKGFYPSDIAVEWESNGQPENNYKTTPPVLDSDGSFFLYSRLTVDKSRWQEGNVFSCSVMHEALHNHYTQKSLSLSLGK

SEQ ID NO: 89 - protein, 220 aa, synthetic construct
DIVMTQSPSSLSVSVGDRVTMTCKSSQSLLNSGNQKNYLTWYQQKPGQPPKLLIYWASTRESGVPDRFSGSGSGTDFTLTISSVQPEDFATYYCQNDYSYPFTFGGGTKLEIKRTVAAPSVFIFPPSDEQLKSGTASVVCLLNNFYPREAKVQWKVDNALQSGNSQESVTEQDSKDSTYSLSSTLTLSKADYEKHKVYACEVTHQGLSSPVTKSFNRGEC

SEQ ID NO: 90 - protein, 220 aa, synthetic construct
DIQMTQSPSSLSASVGDRVTMTCKSSQSLLNSGNQKNYLTWYQQKPGKAPKLLIYWASTRESGVPSRFSGSGSGTDFTLTISSLQPEDFATYYCQNDYSYPFTFGGGTKLEIKRTVAAPSVFIFPPSDEQLKSGTASVVCLLNNFYPREAKVQWKVDNALQSGNSQESVTEQDSKDSTYSLSSTLTLSKADYEKHKVYACEVTHQGLSSPVTKSFNRGEC

SEQ ID NO: 91 - protein, 220 aa, synthetic construct
DIQMTQSPSSLSASVGDRVTITCRSSQSLLNSGNQKNYLTWYQQKPGKAPKLLIYWASTRESGVPSRFSGSGSGTDFTLTISSLQPEDFATYYCQNDYSYPFTFGGGTKLEIKRTVAAPSVFIFPPSDEQLKSGTASVVCLLNNFYPREAKVQWKVDNALQSGNSQESVTEQDSKDSTYSLSSTLTLSKADYEKHKVYACEVTHQGLSSPVTKSFNRGEC

SEQ ID NO: 92 - protein, 449 aa, synthetic construct
QVQLVQSGAEVKKPGASVKLSCKASGYTFTSYWMHWVRQRPGQGLEWIGMIHPNSGSTNYNEKFKSKATLTVDKSTSTAYMELSSLRSEDTAVYYCARRYYGSISPDYWGQGTTVTVSSASTKGPSVFPLAPSSKSTSGGTAALGCLVKDYFPEPVTVSWNSGALTSGVHTFPAVLQSSGLYSLSSVVTVPSSSLGTQTYICNVNHKPSNTKVDKKVEPKSCDKTHTCPPCPAPELLGGPSVFLFPPKPKDTLMISRTPEVTCVVVDVSHEDPEVKFNWYVDGVEVHNAKTKPREEQYNSTYRVVSVLTVLHQDWLNGKEYKCKVSNKALPAPIEKTISKAKGQPREPQVYTLPPSRDELTKNQVSLTCLVKGFYPSDIAVEWESNGQPENNYKTTPPVLDSDGSFFLYSKLTVDKSRWQQGNVFSCSVMHEALHNHYTQKSLSLSPGK

SEQ ID NO: 93 - protein, 449 aa, synthetic construct
QVQLVQSGAEVKKPGASVKLSCKASGYTFTSYWMHWVRQAPGQGLEWIGMIHPNSGSTNYNEKFKSRATLTVDTSTSTAYMELSSLRSEDTAVYYCARRYYGSISPDYWGQGTTVTVSSASTKGPSVFPLAPSSKSTSGGTAALGCLVKDYFPEPVTVSWNSGALTSGVHTFPAVLQSSGLYSLSSVVTVPSSSLGTQTYICNVNHKPSNTKVDKKVEPKSCDKTHTCPPCPAPELLGGPSVFLFPPKPKDTLMISRTPEVTCVVVDVSHEDPEVKFNWYVDGVEVHNAKTKPREEQYNSTYRVVSVLTVLHQDWLNGKEYKCKVSNKALPAPIEKTISKAKGQPREPQVYTLPPSRDELTKNQVSLTCLVKGFYPSDIAVEWESNGQPENNYKTTPPVLDSDGSFFLYSKLTVDKSRWQQGNVFSCSVMHEALHNHYTQKSLSLSPGK

SEQ ID NO: 94 - protein, 449 aa, synthetic construct
QVQLVQSGAEVKKPGASVKVSCKASGYTFTSYWMHWVRQAPGQGLEWIGMIHPNSGSTNYNEKFKSRVTMTVDTSTSTAYMELSSLRSEDTAVYYCARRYYGSISPDYWGQGTTVTVSSASTKGPSVFPLAPSSKSTSGGTAALGCLVKDYFPEPVTVSWNSGALTSGVHTFPAVLQSSGLYSLSSVVTVPSSSLGTQTYICNVNHKPSNTKVDKKVEPKSCDKTHTCPPCPAPELLGGPSVFLFPPKPKDTLMISRTPEVTCVVVDVSHEDPEVKFNWYVDGVEVHNAKTKPREEQYNSTYRVVSVLTVLHQDWLNGKEYKCKVSNKALPAPIEKTISKAKGQPREPQVYTLPPSRDELTKNQVSLTCLVKGFYPSDIAVEWESNGQPENNYKTTPPVLDSDGSFFLYSKLTVDKSRWQQGNVFSCSVMHEALHNHYTQKSLSLSPGK

SEQ ID NO: 95 - protein, 449 aa, synthetic construct
QVQLVQSGAEVKKPGASVKVSCKASGYTFTSYWMHWVRQAPGQGLEWMGMIHPNSGSTNYNEKFKSRVTMTVDTSTSTVYMELSSLRSEDTAVYYCARRYYGSISPDYWGQGTTVTVSSASTKGPSVFPLAPSSKSTSGGTAALGCLVKDYFPEPVTVSWNSGALTSGVHTFPAVLQSSGLYSLSSVVTVPSSSLGTQTYICNVNHKPSNTKVDKKVEPKSCDKTHTCPPCPAPELLGGPSVFLFPPKPKDTLMISRTPEVTCVVVDVSHEDPEVKFNWYVDGVEVHNAKTKPREEQYNSTYRVVSVLTVLHQDWLNGKEYKCKVSNKALPAPIEKTISKAKGQPREPQVYTLPPSRDELTKNQVSLTCLVKGFYPSDIAVEWESNGQPENNYKTTPPVLDSDGSFFLYSKLTVDKSRWQQGNVFSCSVMHEALHNHYTQKSLSLSPGK

SEQ ID NO: 96 - protein, 449 aa, synthetic construct
QVQLVQSGAEVKKPGASVKVSCKASGYTFTSYWMHWVRQAPGQGLEWMGMIHPNSGSTNYAQKFQGRVTMTRDTSTSTVYMELSSLRSEDTAVYYCARRYYGSISPDYWGQGTTVTVSSASTKGPSVFPLAPSSKSTSGGTAALGCLVKDYFPEPVTVSWNSGALTSGVHTFPAVLQSSGLYSLSSVVTVPSSSLGTQTYICNVNHKPSNTKVDKKVEPKSCDKTHTCPPCPAPELLGGPSVFLFPPKPKDTLMISRTPEVTCVVVDVSHEDPEVKFNWYVDGVEVHNAKTKPREEQYNSTYRVVSVLTVLHQDWLNGKEYKCKVSNKALPAPIEKTISKAKGQPREPQVYTLPPSRDELTKNQVSLTCLVKGFYPSDIAVEWESNGQPENNYKTTPPVLDSDGSFFLYSKLTVDKSRWQQGNVFSCSVMHEALHNHYTQKSLSLSPGK

SEQ ID NO: 97 - protein, 446 aa, synthetic construct
QVQLVQSGAEVKKPGASVKLSCKASGYTFTSYWMHWVRQRPGQGLEWIGMIHPNSGSTNYNEKFKSKATLTVDKSTSTAYMELSSLRSEDTAVYYCARRYYGSISPDYWGQGTTVTVSSASTKGPSVFPLAPCSRSTSESTAALGCLVKDYFPEPVTVSWNSGALTSGVHTFPAVLQSSGLYSLSSVVTVPSSSLGTKTYTCNVDHKPSNTKVDKRVESKYGPPCPPCPAPEFLGGPSVFLFPPKPKDTLMISRTPEVTCVVVDVSQEDPEVQFNWYVDGVEVHNAKTKPREEQFNSTYRVVSVLTVLHQDWLNGKEYKCKVSNKGLPSSIEKTISKAKGQPREPQVYTLPPSQEEMTKNQVSLTCLVKGFYPSDIAVEWESNGQPENNYKTTPPVLDSDGSFFLYSRLTVDKSRWQEGNVFSCSVMHEALHNHYTQKSLSLSLGK

SEQ ID NO: 98 - protein, 446 aa, synthetic construct
QVQLVQSGAEVKKPGASVKLSCKASGYTFTSYWMHWVRQAPGQGLEWIGMIHPNSGSTNYNEKFKSRATLTVDTSTSTAYMELSSLRSEDTAVYYCARRYYGSISPDYWGQGTTVTVSSASTKGPSVFPLAPCSRSTSESTAALGCLVKDYFPEPVTVSWNSGALTSGVHTFPAVLQSSGLYSLSSVVTVPSSSLGTKTYTCNVDHKPSNTKVDKRVESKYGPPCPPCPAPEFLGGPSVFLFPPKPKDTLMISRTPEVTCVVVDVSQEDPEVQFNWYVDGVEVHNAKTKPREEQFNSTYRVVSVLTVLHQDWLNGKEYKCKVSNKGLPSSIEKTISKAKGQPREPQVYTLPPSQEEMTKNQVSLTCLVKGFYPSDIAVEWESNGQPENNYKTTPPVLDSDGSFFLYSRLTVDKSRWQEGNVFSCSVMHEALHNHYTQKSLSLSLGK

SEQ ID NO: 99 - protein, 446 aa, synthetic construct
QVQLVQSGAEVKKPGASVKVSCKASGYTFTSYWMHWVRQAPGQGLEWIGMIHPNSGSTNYNEKFKSRVTMTVDTSTSTAYMELSSLRSEDTAVYYCARRYYGSISPDYWGQGTTVTVSSASTKGPSVFPLAPCSRSTSESTAALGCLVKDYFPEPVTVSWNSGALTSGVHTFPAVLQSSGLYSLSSVVTVPSSSLGTKTYTCNVDHKPSNTKVDKRVESKYGPPCPPCPAPEFLGGPSVFLFPPKPKDTLMISRTPEVTCVVVDVSQEDPEVQFNWYVDGVEVHNAKTKPREEQFNSTYRVVSVLTVLHQDWLNGKEYKCKVSNKGLPSSIEKTISKAKGQPREPQVYTLPPSQEEMTKNQVSLTCLVKGFYPSDIAVEWESNGQPENNYKTTPPVLDSDGSFFLYSRLTVDKSRWQEGNVFSCSVMHEALHNHYTQKSLSLSLGK

SEQ ID NO: 100 - protein, 446 aa, synthetic construct
QVQLVQSGAEVKKPGASVKVSCKASGYTFTSYWMHWVRQAPGQGLEWMGMIHPNSGSTNYNEKFKSRVTMTVDTSTSTVYMELSSLRSEDTAVYYCARRYYGSISPDYWGQGTTVTVSSASTKGPSVFPLAPCSRSTSESTAALGCLVKDYFPEPVTVSWNSGALTSGVHTFPAVLQSSGLYSLSSVVTVPSSSLGTKTYTCNVDHKPSNTKVDKRVESKYGPPCPPCPAPEFLGGPSVFLFPPKPKDTLMISRTPEVTCVVVDVSQEDPEVQFNWYVDGVEVHNAKTKPREEQFNSTYRVVSVLTVLHQDWLNGKEYKCKVSNKGLPSSIEKTISKAKGQPREPQVYTLPPSQEEMTKNQVSLTCLVKGFYPSDIAVEWESNGQPENNYKTTPPVLDSDGSFFLYSRLTVDKSRWQEGNVFSCSVMHEALHNHYTQKSLSLSLGK

SEQ ID NO: 101 - protein, 446 aa, synthetic construct
QVQLVQSGAEVKKPGASVKVSCKASGYTFTSYWMHWVRQAPGQGLEWMGMIHPNSGSTNYAQKFQGRVTMTRDTSTSTVYMELSSLRSEDTAVYYCARRYYGSISPDYWGQGTTVTVSSASTKGPSVFPLAPCSRSTSESTAALGCLVKDYFPEPVTVSWNSGALTSGVHTFPAVLQSSGLYSLSSVVTVPSSSLGTKTYTCNVDHKPSNTKVDKRVESKYGPPCPPCPAPEFLGGPSVFLFPPKPKDTLMISRTPEVTCVVVDVSQEDPEVQFNWYVDGVEVHNAKTKPREEQFNSTYRVVSVLTVLHQDWLNGKEYKCKVSNKGLPSSIEKTISKAKGQPREPQVYTLPPSQEEMTKNQVSLTCLVKGFYPSDIAVEWESNGQPENNYKTTPPVLDSDGSFFLYSRLTVDKSRWQEGNVFSCSVMHEALHNHYTQKSLSLSLGK

SEQ ID NO: 102 - protein, 113 aa, synthetic construct
DIVMTQSPSSLTVTAGEKVTMSCKSSQSLFNSGNQKNYLTWYQQKPGQPPKLLIYWASTRESGVPDRFTGSGSGTDFTLTISSVQAEDLAVYFCQNDYSYPLTFGAGTKLELK

SEQ ID NO: 103 - protein, 115 aa, synthetic construct
EVQLQQSGPELVRPGASVKMSCKASGYTFTDYNMHWVKQSHGKSLEWIGYINPNNGGTSYNQKFKGKATLTVNKSSSTAYMELRSLTSEDSAVYYCVTTRYLAVWGTGTTVTVSS

SEQ ID NO: 104 - protein, 113 aa, synthetic construct
DIVMTQSPSSLSVTAGEKVTMSCKSSQSLLNSGNQKNYLTWYQQKPGQPPKLLIYWASTRESGVPDRFTGSGSGTDFTLTISSVQAEDLAVYYCQNDYSYPFTFGSGTKLEIK

SEQ ID NO: 105 - protein, 119 aa, synthetic construct
QVQLQQPGSELVKPGASVKLSCKASGYTFTSYWMHWVKQRPGQGLEWIGMIHPNSGSTNYNEKFKSKATLTVDKSSSTAYMQLSSLTSEDSAVYYCARRYYGSISPDYWGQGTTLTVSS

SEQ ID NO: 106 - protein, 24 aa, synthetic construct
IYIWAPLAGTCGVLLLSLVITLYC

SEQ ID NO: 107 - protein, 24 aa, synthetic construct
FWLPIGCAAFVVVCILGCILICWL

SEQ ID NO: 108 - protein, 26 aa, synthetic construct
VAAILGLGLVLGLLGPLAILLALYLL

SEQ ID NO: 109 - protein, 42 aa, synthetic construct
KRGRKKLLYIFKQPFMRPVQTTQEEDGCSCRFPEEEEGGCEL

SEQ ID NO: 110 - protein, 38 aa, synthetic construct
CWLTKKKYSSSVHDPNGEYMFMRAVNTAKKSRLTDVTL

SEQ ID NO: 111 - protein, 45 aa, synthetic construct
TTTPAPRPPTPAPTIASQPLSLRPEACRPAAGGAVHTRGLDFACD

SEQ ID NO: 112 - protein, 113 aa, synthetic construct
RVKFSRSADAPAYQQGQNQLYNELNLGRREEYDVLDKRRGRDPEMGGKPQRRKNPQEGLYNELQKDKMAEAYSEIGMKGERRRGKGHDGLYQGLSTATKDTYDALHMQALPPR